European Patent Application EP 4 696 706 A1, published February 18, 2026. Title: 세포의 줄기세포능 유도 인자 및 이를 이용하여 세포의 줄기세포능을 증가 또는 유지시키는 방법. Applicant: 의료법인 성광의료재단. Application KR. The sequence listing filed with the application follows.

SEQUENCE LISTING (7 sequences)

SEQ ID NO: 1 - protein, 145 aa, synthetic construct
MEDLQNQFQKELAEQRAELEKIFQDKNQAERALRNLESHHQAAIEKLREDLQSEHGRCLEDLEFKFKESEKEKQLELENLQASYEDLKAQSQEEIRRLWSQLDSARTSRQELSELHEQLLARTSRVEDLEQLKQREKTQHESELE

SEQ ID NO: 2 - DNA, 435 bp, synthetic construct
  source 1..435: mol_type = other DNA
atggaggatttacaaaaccagtttcagaaagaattggcagaacagagagctgagttggagaagatttttcaagacaaaaaccaggctgaacgggcccttaggaacctggagagtcatcatcaagcagccattgagaagttacgtgaagacctgcagtccgagcacggccggtgtttagaagacttggagttcaagttcaaagagagcgagaaagaaaaacagctggagttagagaatcttcaagcatcatatgaagacctgaaggcacaatcacaagaagagatcaggcgcttgtggtcccagcttgattctgccaggaccagtagacaggaattgagtgagctacatgagcaactcctggcgcgcacctctcgtgtggaagatttagaacagctgaagcagcgagaaaaaacccagcatgagtccgaactggag

SEQ ID NO: 3 - protein, 3336 aa, synthetic construct [sequence omitted]

SEQ ID NO: 4 - DNA, 19 bp, synthetic construct
  source 1..19: mol_type = other DNA
gctgaacgggcccttagga

SEQ ID NO: 5 - DNA, 20 bp, synthetic construct
  source 1..20: mol_type = other DNA
cctgtctactggtcctggca

SEQ ID NO: 6 - DNA, 20 bp, synthetic construct
  source 1..20: mol_type = other DNA
gtaacccgttgaaccccatt

SEQ ID NO: 7 - DNA, 20 bp, synthetic construct
  source 1..20: mol_type = other DNA
ccatccaatcggtagtagcg